European Patent Specification EP 3 682 033 B1, published December 3, 2025. Title: Single-Molecule Phenotyping and Sequencing of Nucleic Acid Molecules. Applicant: Oxford University Innovation Limited. The sequence listing filed with the application follows.

SEQUENCE LISTING (24 sequences)

SEQ ID NO: 1 - DNA, 22 bp, Unknown
  Unknown
aaatgtgatctagatcacattt

SEQ ID NO: 2 - DNA, 78 bp, Unknown
  Unknown
ctgctgcctcaggctcataagagcctgaggcagcagattatcgacggtggatgtatggtaatgggacgaagaatgagg

SEQ ID NO: 3 - DNA, 27 bp, Unknown
  Unknown
cctcattcttcgtcccattaccataca

SEQ ID NO: 4 - DNA, 65 bp, Unknown
  Unknown
cagtcaagagcctgaggcagcagattatcgacggtggatgtatggtaatgggacgaagaatgagg

SEQ ID NO: 5 - DNA, 29 bp, Unknown
  Unknown
gataatctgctgcctcaggctcttgactg

SEQ ID NO: 6 - DNA, 30 bp, Unknown
  Unknown
cgataatctgctgcctcaggctcttgactg

SEQ ID NO: 7 - DNA, 32 bp, Unknown
  Unknown
gtcgataatctgctgcctcaggctcttgactg

SEQ ID NO: 8 - DNA, 65 bp, Unknown
  Unknown
cagtcaagagcctgaggcagcagattatcgacggaggatgtatggtaatgggacgaagaatgagg

SEQ ID NO: 9 - DNA, 31 bp, Unknown
  Unknown
tcgataatctgctgcctcaggctcttgactg

SEQ ID NO: 10 - DNA, 65 bp, Unknown
  Unknown
cagtcaagagcctgaggcagcagattatcgaataatattgtatggtaatgggacgaagaatgagg

SEQ ID NO: 11 - DNA, 25 bp, Unknown
  Unknown
atctgctgcctcaggctcttgactg

SEQ ID NO: 12 - DNA, 12 bp, Unknown
  Unknown
tccaccgtcgat

SEQ ID NO: 13 - DNA, 13 bp, Unknown
  Unknown
  n (10)..(13): any base or universal base
  misc_feature (10)..(13): n is a, c, g, or t
tccaccgtcnnnn

SEQ ID NO: 14 - DNA, 13 bp, Unknown
  Unknown
  n (10)..(13): any base or universal base
  misc_feature (10)..(13): n is a, c, g, or t
tccaccgtgnnnn

SEQ ID NO: 15 - DNA, 45 bp, Unknown
  Unknown
taaatctaaagtaacataaggtaacataacgtaagctcattcgcg

SEQ ID NO: 16 - DNA, 45 bp, Unknown
  Unknown
cgcgaatgagcttacgttatgttaccttatgttactttagattta

SEQ ID NO: 17 - DNA, 73 bp, Unknown
  Unknown
cccactgccgaatgtgagttagctcactcacgaaaaaccactgtcgaaaaagctctacgggctctggcgtcgg

SEQ ID NO: 18 - DNA, 68 bp, Unknown
  Unknown
ccgacgccagagcccgtagagccgacagtggcgtgagtgagctaactcacattcgaaaaagcagtggg

SEQ ID NO: 19 - DNA, 49 bp, Unknown
  Unknown
gtgcctaaaatgtgatctagatcacatttattgcgtagagctcactgcc

SEQ ID NO: 20 - DNA, 49 bp, Unknown
  Unknown
ggcagtgagctctacgcaataaatgtgatctagatcacattttaggcac

SEQ ID NO: 21 - DNA, 49 bp, Unknown
  Unknown
gtgcctaaaatgtgatctagatcagatttattgcgtagagctcactgcc

SEQ ID NO: 22 - DNA, 49 bp, Unknown
  Unknown
ggcagtgagctctacgcaataaatctgatctagatcacattttaggcac

SEQ ID NO: 23 - DNA, 20 bp, Unknown
  Unknown
ggcagtgagctctacgcaat

SEQ ID NO: 24 - DNA, 20 bp, Unknown
  Unknown
ctagatcacattttaggcac